European Patent Specification EP 3 986 438 B1, published April 16, 2025. Title: P53 ACTIVATOR PEPTIDOMIMETIC MACROCYCLES. Applicant: Merck Sharp & Dohme Corp. MSD International GmbH (Singapore Branch) Agency For Science, Technology And Research Aronica, Pietro Brown, Christopher J Ferrer, Fernando J Johannes, Charles W Kannan, Srinivasaraghavan Lane, David P Partridge, Anthony W Sawyer, Tomi K Tan, Yaw Sing Verma, Chandra S Yuen, Tsz Ying. The sequence listing filed with the application follows.

SEQUENCE LISTING (24 sequences)

SEQ ID NO: 1 - protein, 12 aa, Artificial Sequence
  D-DPMI-delta
  MISC_FEATURE (1)..(12): Xaa1-Xaa12 all alpha-amino acids thereof have a D configuration
  VARIANT (3)..(3): Xaa3 is 6-F-Trp
  VARIANT (7)..(7): Xaa7 is p-CF3-Phe
  MISC_FEATURE (12)..(12): Xaa12 optionally has a C-terminal amide
TAXYANXEKLLR

SEQ ID NO: 2 - protein, 12 aa, Artificial Sequence
  D-PMI-delta(1-5)
  VARIANT (1)..(1): Xaa1 is (R)-2-(4'-pentenyl)-alanine
  MISC_FEATURE (1)..(12): Xaa1-Xaa12 all alpha-amino acids thereof have a D configuration
  MISC_FEATURE (1)..(1): Xaa1 optionally has a N-terminal acyl
  VARIANT (3)..(3): Xaa3 is 6-F-Trp
  VARIANT (5)..(5): Xaa5 is (R)-2-(4'-pentenyl)-alanine
  VARIANT (7)..(7): Xaa7 is p-CF3-Phe
  MISC_FEATURE (12)..(12): Xaa12 optionally has a C-terminal amide
XAXYXNXEKLLR

SEQ ID NO: 3 - protein, 12 aa, Artificial Sequence
  D-PMI-delta(2-6)
  MISC_FEATURE (1)..(12): Xaa1-Xaa12 all alpha-amino acids thereof have a D configuration
  MISC_FEATURE (1)..(1): Xaa1 optionally has a N-terminal acyl
  VARIANT (2)..(2): Xaa2 is (R)-2-(4'-pentenyl)-alanine
  VARIANT (3)..(3): Xaa3 is 6-F-Trp
  VARIANT (6)..(6): Xaa6 is (R)-2-(4'-pentenyl)-alanine
  VARIANT (7)..(7): Xaa7 is p-CF3-Phe
  MISC_FEATURE (12)..(12): Xaa12 optionally has a C-terminal amide
TXXYAXXEKLLR

SEQ ID NO: 4 - protein, 12 aa, Artificial Sequence
  D-PMI-delta(2-9)
  MISC_FEATURE (1)..(12): Xaa1-Xaa12 all alpha-amino acids thereof have a D configuration
  MISC_FEATURE (1)..(1): Xaa1 optionally has a N-terminal acyl
  VARIANT (2)..(2): Xaa2 is (S)-2-(7'-octenyl)-alanine
  VARIANT (3)..(3): Xaa3 is 6-F-Trp
  VARIANT (7)..(7): Xaa7 is p-CF3-Phe
  VARIANT (9)..(9): Xaa9 is (R)-2-(4'-pentenyl)-alanine
  MISC_FEATURE (12)..(12): Xaa12 optionally has a C-terminal amide
TXXYANXEXLLR

SEQ ID NO: 5 - protein, 12 aa, Artificial Sequence
  D-PMI-delta(5-9)
  MISC_FEATURE (1)..(12): Xaa1-Xaa12 all alpha-amino acids thereof have a D configuration
  MISC_FEATURE (1)..(1): Xaa1 optionally has a N-terminal acyl
  VARIANT (3)..(3): Xaa3 is 6-F-Trp
  VARIANT (5)..(5): Xaa5 is (R)-2-(4'-pentenyl)-alanine
  VARIANT (7)..(7): Xaa7 is p-CF3-Phe
  VARIANT (9)..(9): Xaa9 is (R)-2-(4'-pentenyl)-alanine
  MISC_FEATURE (12)..(12): Xaa12 optionally has a C-terminal amide
TAXYXNXEXLLR

SEQ ID NO: 6 - protein, 12 aa, Artificial Sequence
  D-PMI-delta(5-12)
  MISC_FEATURE (1)..(12): Xaa1-Xaa12 all alpha-amino acids thereof have a D configuration
  MISC_FEATURE (1)..(1): Xaa1 optionally has a N-terminal acyl
  VARIANT (3)..(3): Xaa3 is 6-F-Trp
  VARIANT (5)..(5): Xaa5 is (S)-2-(7'-octenyl)-alanine
  VARIANT (7)..(7): Xaa7 is p-CF3-Phe
  VARIANT (12)..(12): Xaa12 is (R)-2-(4'-pentenyl)-alanine
TAXYXNXEKLLX

SEQ ID NO: 7 - protein, 12 aa, Artificial Sequence
  D-PMI-delta(6-10)
  MISC_FEATURE (1)..(12): Xaa1-Xaa12 all alpha-amino acids thereof have a D configuration
  MISC_FEATURE (1)..(1): Xaa1 optionally has a N-terminal acyl
  VARIANT (3)..(3): Xaa3 is 6-F-Trp
  VARIANT (6)..(6): Xaa6 is (R)-2-(4'-pentenyl)-alanine
  VARIANT (7)..(7): Xaa7 is p-CF3-Phe
  VARIANT (10)..(10): Xaa10 is (R)-2-(4'-pentenyl)-alanine
  MISC_FEATURE (12)..(12): Xaa12 optionally has a C-terminal amide
TAXYAXXEKXLR

SEQ ID NO: 8 - protein, 12 aa, Artificial Sequence
  D-PMI-delta(1,5,12)
  VARIANT (1)..(1): Xaa1 is (R)-2-(4'-pentenyl)-alanine
  MISC_FEATURE (1)..(12): Xaa1-Xaa12 all alpha-amino acids thereof have a D configuration
  MISC_FEATURE (1)..(1): Xaa1 optionally has a N-terminal acyl
  VARIANT (3)..(3): Xaa3 is 6-F-Trp
  VARIANT (5)..(5): Xaa5 is 2,2-(4'-penenyl)-glycine
  VARIANT (7)..(7): Xaa7 is p-CF3-Phe
  VARIANT (12)..(12): Xaa12 is (R)-2-(7'-octenyl)-alanine
  MISC_FEATURE (12)..(12): Xaa12 optionally has a C-terminal amide
XAXYXNXEKLLX

SEQ ID NO: 9 - protein, 12 aa, Artificial Sequence
  D-PMI-delta(1-5, 9-12)
  VARIANT (1)..(1): Xaa1 is (R)-2-(4'-pentenyl)-alanine
  MISC_FEATURE (1)..(12): Xaa1-Xaa12 all alpha-amino acids thereof have a D configuration
  MISC_FEATURE (1)..(1): Xaa1 optionally has a N-terminal acyl
  VARIANT (3)..(3): Xaa3 is 6-F-Trp
  VARIANT (5)..(5): Xaa5 is (R)-2-(4'-pentenyl)-alanine
  VARIANT (7)..(7): Xaa7 is p-CF3-Phe
  VARIANT (9)..(9): Xaa9 is (S)-2-(4'-pentenyl)-alanine
  VARIANT (12)..(12): Xaa12 is (R)-2-(7'-octenyl)-alanine
  MISC_FEATURE (12)..(12): Xaa12 optionally has a C-terminal amide
XAXYXNXEXLLX

SEQ ID NO: 10 - protein, 125 aa, Artificial Sequence
  N-terminal domain of MDM2
  MISC_FEATURE (1)..(125)
MCNTNMSVPTDGAVTTSQIPASEQETLVRPKPLLLKLLKSVGAQKDTYTMKEVLFYLGQYIMTKRLYDEKQQHIVYCSNDLLGDLFGVPSFSVKEHRKIYTMIYRNLVVVNQQESSDSGTSVSEN

SEQ ID NO: 11 - protein, 125 aa, Artificial Sequence
  N-terminal domain of MDM4 (MDMX)
  MISC_FEATURE (1)..(125)
MTSFSTSAQCSTSDSACRISPGQINQVRPKLPLLKILHAAGAQGEMFTVKEVMHYLGQYIMVKQLYDQQEQHMVYCGGDLLGELLGRQSFSVKDPSPLYDMLRKNLVTLATATTDAAQTLALAQD

SEQ ID NO: 12 - protein, 379 aa, Artificial Sequence
  Human MDM2 1-125 sequence
  MISC_FEATURE (1)..(379): All alpha-amino acids have an L configuration
MSDKIIHSPILGYWKIKGLVQPTRLLLEYLEEKYEEHLYERDEGDKWRNKKFELGLEFPNLPYYIDGDVKLTQSMAIIRYIADKHNMLGGCPKERAEISMLEGAVLDIRYGVSRIAYSKDFETLKVDFLSKLPEMLKMFEDRLCHKTYLNGDHVTHPDFMLYDALDVVLYMDPMCLDAFPKLVCFKKRIEAIPQIDKYLKSSKYIAWPLQGWQATFGGGDHPPKLEVLFQGHMHHHHHHSSGVDLGTENLYFQGMCNTNMSVPTDGAVTTSQIPASEQETLVRPKPLLLKLLKSVGAQKDTYTMKEVLFYLGQYIMTKRLYDEKQQHIVYCSNDLLGDLFGVPSFSVKEHRKIYTMIYRNLVVVNQQESSDSGTSVSEN

SEQ ID NO: 13 - protein, 7 aa, Artificial Sequence
  TV cleavage site
  MISC_FEATURE (1)..(7): All alpha-amino acids have an L configuration
ENLYFQS

SEQ ID NO: 14 - protein, 7 aa, Artificial sequence
  TV cleavage site with S7G substitution
  MISC_FEATURE (1)..(7): All alpha-amino acids have an L configuration
ENLYFQG

SEQ ID NO: 15 - protein, 393 aa, Homo spaiens [sequence omitted]

SEQ ID NO: 16 - protein, 12 aa, Artificial Sequence
  D-PMI-delta variant
  VARIANT (1)..(1): Xaa1 is an alpha-amino or an alpha,alpha-disubstituted amino acid
  MISC_FEATURE (1)..(12): Xaa1-Xaa12 all alpha-amino acids thereof have a D configuration
  MISC_FEATURE (1)..(1): Xaa1 optionally has a N-terminal acyl
  VARIANT (3)..(3): Xaa3 is 6-F-Trp
  VARIANT (5)..(5): Xaa5 is an alpha-amino or an alpha,alpha-disubstituted amino acid
  VARIANT (7)..(7): Xaa7 is p-CF3-Phe
  VARIANT (9)..(9): Xaa9 is an alpha-amino or an alpha,alpha-disubstituted amino acid
  VARIANT (12)..(12): Xaa12 is an alpha-amino or an alpha,alpha-disubstituted amino acid
  MISC_FEATURE (12)..(12): Xaa12 optionally has a C-terminal amide
XAXYXNXEXLLX

SEQ ID NO: 17 - protein, 12 aa, Artificial Sequence
  D-PMI-delta(1-5)
  VARIANT (1)..(1): Xaa1 is (R)-2-(4'-pentenyl)-alanine
  MISC_FEATURE (1)..(12): Xaa1-Xaa12 all alpha-amino acids thereof have a D configuration
  VARIANT (3)..(3): Xaa3 is 6-F-Trp
  VARIANT (5)..(5): Xaa5 is (R)-2-(4'-pentenyl)-alanine
  VARIANT (7)..(7): Xaa7 is p-CF3-Phe
  MISC_FEATURE (12)..(12): Xaa12 has a C-terminal amide
XAXYXNXEKLLR

SEQ ID NO: 18 - protein, 12 aa, Artificial Sequence
  D-PMI-delta(2-6)
  MISC_FEATURE (1)..(12): Xaa1-Xaa12 all alpha-amino acids thereof have a D configuration
  VARIANT (2)..(2): Xaa2 is (R)-2-(4'-pentenyl)-alanine
  VARIANT (3)..(3): Xaa3 is 6-F-Trp
  VARIANT (6)..(6): Xaa6 is (R)-2-(4'-pentenyl)-alanine
  VARIANT (7)..(7): Xaa7 is p-CF3-Phe
  MISC_FEATURE (12)..(12): Xaa12 has a C-terminal amide
TXXYAXXEKLLR

SEQ ID NO: 19 - protein, 12 aa, Artificial Sequence
  D-PMI-delta(2-9)
  MISC_FEATURE (1)..(12): Xaa1-Xaa12 all alpha-amino acids thereof have a D configuration
  VARIANT (2)..(2): Xaa2 is (S)-2-(7'-octenyl)-alanine
  VARIANT (3)..(3): Xaa3 is 6-F-Trp
  VARIANT (7)..(7): Xaa7 is p-CF3-Phe
  VARIANT (9)..(9): Xaa9 is (R)-2-(4'-pentenyl)-alanine
  MISC_FEATURE (12)..(12): Xaa12 has a C-terminal amide
TXXYANXEXLLR

SEQ ID NO: 20 - protein, 12 aa, Artificial Sequence
  D-PMI-delta(5-9)
  MISC_FEATURE (1)..(12): Xaa1-Xaa12 all alpha-amino acids thereof have a D configuration
  VARIANT (3)..(3): Xaa3 is 6-F-Trp
  VARIANT (5)..(5): Xaa5 is (R)-2-(4'-pentenyl)-alanine
  VARIANT (7)..(7): Xaa7 is p-CF3-Phe
  VARIANT (9)..(9): Xaa9 is (R)-2-(4'-pentenyl)-alanine
  MISC_FEATURE (12)..(12): Xaa12 has a C-terminal amide
TAXYXNXEXLLR

SEQ ID NO: 21 - protein, 12 aa, Artificial Sequence
  D-PMI-delta(5-12)
  MISC_FEATURE (1)..(12): Xaa1-Xaa12 all alpha-amino acids thereof have a D configuration
  VARIANT (3)..(3): Xaa3 is 6-F-Trp
  VARIANT (5)..(5): Xaa5 is (S)-2-(7'-octenyl)-alanine
  VARIANT (7)..(7): Xaa7 is p-CF3-Phe
  VARIANT (12)..(12): Xaa12 is (R)-2-(4'-pentenyl)-alanine
  MISC_FEATURE (12)..(12): Xaa12 has a C-terminal amide
TAXYXNXEKLLX

SEQ ID NO: 22 - protein, 12 aa, Artificial Sequence
  D-PMI-delta(6-10)
  MISC_FEATURE (1)..(12): Xaa1-Xaa12 all alpha-amino acids thereof have a D configuration
  MISC_FEATURE (1)..(12): Xaa12 has a C-terminal amide
  VARIANT (3)..(3): Xaa3 is 6-F-Trp
  VARIANT (6)..(6): Xaa6 is (R)-2-(4'-pentenyl)-alanine
  VARIANT (7)..(7): Xaa7 is p-CF3-Phe
  VARIANT (10)..(10): Xaa10 is (R)-2-(4'-pentenyl)-alanine
TAXYAXXEKXLR

SEQ ID NO: 23 - protein, 12 aa, Artificial Sequence
  D-PMI-delta(1,5,12)
  VARIANT (1)..(1): Xaa1 is (R)-2-(4'-pentenyl)-alanine
  VARIANT (3)..(3): Xaa3 is 6-F-Trp
  VARIANT (5)..(5): Xaa5 is 2,2-(4'-penenyl)-glycine
  VARIANT (7)..(7): Xaa7 is p-CF3-Phe
  VARIANT (12)..(12): Xaa12 is (R)-2-(7'-octenyl)-alanine
  MISC_FEATURE (12)..(12): Xaa1-Xaa12 all alpha-amino acids thereof have a D configuration
  MISC_FEATURE (12)..(12): Xaa12 has a C-terminal amide
XAXYXNXEKLLX

SEQ ID NO: 24 - protein, 12 aa, Artificial Sequence
  D-PMI-delta(1-5, 9-12)
  VARIANT (1)..(1): Xaa1 is (R)-2-(4'-pentenyl)-alanine
  MISC_FEATURE (1)..(12): Xaa1-Xaa12 all alpha-amino acids thereof have a D configuration
  VARIANT (3)..(3): Xaa3 is 6-F-Trp
  VARIANT (5)..(5): Xaa5 is (R)-2-(4'-pentenyl)-alanine
  VARIANT (7)..(7): Xaa7 is p-CF3-Phe
  VARIANT (9)..(9): Xaa9 is (S)-2-(4'-pentenyl)-alanine
  VARIANT (12)..(12): Xaa12 is (R)-2-(7'-octenyl)-alanine
  MISC_FEATURE (12)..(12): Xaa12 has a C-terminal amide
XAXYXNXEXLLX